European Patent Application EP 4 592 382 A1, published July 30, 2025. Title: High-performance matured intestinal organoid regenerative medicine derived from pluripotent stem cells. Applicant: 한국생명공학연구원. The sequence listing filed with the application follows.

SEQUENCE LISTING (64 sequences)

SEQ ID NO: 1 - DNA, 19 bp, synthetic construct
  source 1..19: mol_type = other DNA
gaaggtgaaggtcggagtc

SEQ ID NO: 2 - DNA, 20 bp, synthetic construct
  source 1..20: mol_type = other DNA
gaagatggtgatgggatttc

SEQ ID NO: 3 - DNA, 20 bp, synthetic construct
  source 1..20: mol_type = other DNA
agccagatcactgctgaggt

SEQ ID NO: 4 - DNA, 20 bp, synthetic construct
  source 1..20: mol_type = other DNA
tggacaggtgttcctccttc

SEQ ID NO: 5 - DNA, 20 bp, synthetic construct
  source 1..20: mol_type = other DNA
tggcctacacaagcatctgg

SEQ ID NO: 6 - DNA, 20 bp, synthetic construct
  source 1..20: mol_type = other DNA
taactggctgctgtaacggg

SEQ ID NO: 7 - DNA, 20 bp, synthetic construct
  source 1..20: mol_type = other DNA
tgacctcaacgatgcatttc

SEQ ID NO: 8 - DNA, 20 bp, synthetic construct
  source 1..20: mol_type = other DNA
ctgtcctggctcttctgctc

SEQ ID NO: 9 - DNA, 20 bp, synthetic construct
  source 1..20: mol_type = other DNA
tgtaggcatcgctcttctca

SEQ ID NO: 10 - DNA, 20 bp, synthetic construct
  source 1..20: mol_type = other DNA
gacaccatctacctcacccg

SEQ ID NO: 11 - DNA, 20 bp, synthetic construct
  source 1..20: mol_type = other DNA
cggatgactgcctcaatggt

SEQ ID NO: 12 - DNA, 20 bp, synthetic construct
  source 1..20: mol_type = other DNA
aaagacgctcccttctgctc

SEQ ID NO: 13 - DNA, 21 bp, synthetic construct
  source 1..21: mol_type = other DNA
aaaaccccaggagcagttaat

SEQ ID NO: 14 - DNA, 20 bp, synthetic construct
  source 1..20: mol_type = other DNA
caaccctctttgcacaagct

SEQ ID NO: 15 - DNA, 20 bp, synthetic construct
  source 1..20: mol_type = other DNA
acctttcccgtggacagagt

SEQ ID NO: 16 - DNA, 23 bp, synthetic construct
  source 1..23: mol_type = other DNA
tggacatattccctcactttgga

SEQ ID NO: 17 - DNA, 20 bp, synthetic construct
  source 1..20: mol_type = other DNA
ggtaaggagaaaccgggaag

SEQ ID NO: 18 - DNA, 20 bp, synthetic construct
  source 1..20: mol_type = other DNA
gcacgtcgacctatggaaat

SEQ ID NO: 19 - DNA, 20 bp, synthetic construct
  source 1..20: mol_type = other DNA
tcctcgcctacaacctcaac

SEQ ID NO: 20 - DNA, 20 bp, synthetic construct
  source 1..20: mol_type = other DNA
gctgggacactccattctct

SEQ ID NO: 21 - DNA, 21 bp, synthetic construct
  source 1..21: mol_type = other DNA
cagaagactgggaacatttga

SEQ ID NO: 22 - DNA, 20 bp, synthetic construct
  source 1..20: mol_type = other DNA
cacacttgaacacgccactt

SEQ ID NO: 23 - DNA, 20 bp, synthetic construct
  source 1..20: mol_type = other DNA
cctttgcaggaaatggactc

SEQ ID NO: 24 - DNA, 20 bp, synthetic construct
  source 1..20: mol_type = other DNA
ggactcacgggtagcacaac

SEQ ID NO: 25 - DNA, 20 bp, synthetic construct
  source 1..20: mol_type = other DNA
gtgcagtcagcacaaagtgg

SEQ ID NO: 26 - DNA, 20 bp, synthetic construct
  source 1..20: mol_type = other DNA
atgcacatccggaatgggtt

SEQ ID NO: 27 - DNA, 20 bp, synthetic construct
  source 1..20: mol_type = other DNA
atctcctgtttgaccggcag

SEQ ID NO: 28 - DNA, 20 bp, synthetic construct
  source 1..20: mol_type = other DNA
gtcgtcagagtcggggtttg

SEQ ID NO: 29 - DNA, 20 bp, synthetic construct
  source 1..20: mol_type = other DNA
tgcggccaaatgttattttc

SEQ ID NO: 30 - DNA, 20 bp, synthetic construct
  source 1..20: mol_type = other DNA
tgcatggtttctgacatcgt

SEQ ID NO: 31 - DNA, 20 bp, synthetic construct
  source 1..20: mol_type = other DNA
cagcccaaagtgtgtgagaa

SEQ ID NO: 32 - DNA, 20 bp, synthetic construct
  source 1..20: mol_type = other DNA
cggtcaaactgcccatactt

SEQ ID NO: 33 - DNA, 21 bp, synthetic construct
  source 1..21: mol_type = other DNA
gagcatgagggaagatgcgac

SEQ ID NO: 34 - DNA, 21 bp, synthetic construct
  source 1..21: mol_type = other DNA
tgaccacaccaactaggatga

SEQ ID NO: 35 - DNA, 20 bp, synthetic construct
  source 1..20: mol_type = other DNA
gctttccatccaggtgtcat

SEQ ID NO: 36 - DNA, 20 bp, synthetic construct
  source 1..20: mol_type = other DNA
accacgaatccatctccaac

SEQ ID NO: 37 - DNA, 20 bp, synthetic construct
  source 1..20: mol_type = other DNA
gctcgagaaggatgtggtcc

SEQ ID NO: 38 - DNA, 20 bp, synthetic construct
  source 1..20: mol_type = other DNA
cgttgtgcatagtcgctgct

SEQ ID NO: 39 - DNA, 20 bp, synthetic construct
  source 1..20: mol_type = other DNA
gcagaaggcctcagcaccta

SEQ ID NO: 40 - DNA, 19 bp, synthetic construct
  source 1..19: mol_type = other DNA
aggttcccagtcgggttca

SEQ ID NO: 41 - DNA, 26 bp, synthetic construct
  source 1..26: mol_type = other DNA
tgggagcggtgaagatggaagggcac

SEQ ID NO: 42 - DNA, 26 bp, synthetic construct
  source 1..26: mol_type = other DNA
tcatgccagcgcccacgtacgacgac

SEQ ID NO: 43 - DNA, 26 bp, synthetic construct
  source 1..26: mol_type = other DNA
cgctttcatggtgtgggctaaggacg

SEQ ID NO: 44 - DNA, 26 bp, synthetic construct
  source 1..26: mol_type = other DNA
tagttggggtggtcctgcatgtgctg

SEQ ID NO: 45 - DNA, 22 bp, synthetic construct
  source 1..22: mol_type = other DNA
ctggagctggagaaggagtttc

SEQ ID NO: 46 - DNA, 24 bp, synthetic construct
  source 1..24: mol_type = other DNA
attttaacctgcctctcagagagc

SEQ ID NO: 47 - DNA, 20 bp, synthetic construct
  source 1..20: mol_type = other DNA
tgctcttcaccaactgcatc

SEQ ID NO: 48 - DNA, 20 bp, synthetic construct
  source 1..20: mol_type = other DNA
ctcaggctcaccagatcctc

SEQ ID NO: 49 - DNA, 20 bp, synthetic construct
  source 1..20: mol_type = other DNA
cgtgaagctggtgaacttgg

SEQ ID NO: 50 - DNA, 20 bp, synthetic construct
  source 1..20: mol_type = other DNA
ggatgtactccacggctgag

SEQ ID NO: 51 - DNA, 22 bp, synthetic construct
  source 1..22: mol_type = other DNA
gagtggacttgtgccgacttca

SEQ ID NO: 52 - DNA, 22 bp, synthetic construct
  source 1..22: mol_type = other DNA
ggtggctggtgcaaagacatag

SEQ ID NO: 53 - DNA, 20 bp, synthetic construct
  source 1..20: mol_type = other DNA
gggggaggttggactgtaat

SEQ ID NO: 54 - DNA, 20 bp, synthetic construct
  source 1..20: mol_type = other DNA
gaataggctcggttcccttc

SEQ ID NO: 55 - DNA, 20 bp, synthetic construct
  source 1..20: mol_type = other DNA
cccacgttttcagagttggt

SEQ ID NO: 56 - DNA, 20 bp, synthetic construct
  source 1..20: mol_type = other DNA
cggctctttcgcttactgtt

SEQ ID NO: 57 - DNA, 20 bp, synthetic construct
  source 1..20: mol_type = other DNA
ttcaatgtcccagccatgta

SEQ ID NO: 58 - DNA, 20 bp, synthetic construct
  source 1..20: mol_type = other DNA
gaaggaatagccacgctcag

SEQ ID NO: 59 - DNA, 24 bp, synthetic construct
  source 1..24: mol_type = other DNA
agaacgtgcaggaggcagaagaat

SEQ ID NO: 60 - DNA, 24 bp, synthetic construct
  source 1..24: mol_type = other DNA
ttccatttcacgcatctggcgttc

SEQ ID NO: 61 - DNA, 20 bp, synthetic construct
  source 1..20: mol_type = other DNA
cagtggctaccaggacaaca

SEQ ID NO: 62 - DNA, 20 bp, synthetic construct
  source 1..20: mol_type = other DNA
ctcagaacccctttgctcag

SEQ ID NO: 63 - DNA, 19 bp, synthetic construct
  source 1..19: mol_type = other DNA
gtggcatcgttgaggagtg

SEQ ID NO: 64 - DNA, 19 bp, synthetic construct
  source 1..19: mol_type = other DNA
cacgtccctctcggacttg